European Patent Application EP 4 545 552 A1, published April 30, 2025. Title: carrier peptide fragment and use thereof. Applicant: TOAGOSEI CO., LTD. The sequence listing filed with the application follows.

SEQUENCE LISTING (3 sequences)

SEQ ID NO: 1 - protein, 13 aa, synthetic construct
  source 1..13: note = synthetic peptide
RKKRNSKRLTRKK

SEQ ID NO: 2 - protein, 13 aa, synthetic construct
  SITE 1: note = D-Arginine
  SITE 4: note = D-Arginine
  SITE 8: note = D-Arginine
  SITE 11: note = D-Arginine
RKKRNSKRLTRKK

SEQ ID NO: 3 - protein, 13 aa, synthetic construct
  SITE 2..3: note = D-Lysine
  SITE 7: note = D-Lysine
  SITE 12..13: note = D-Lysine
RKKRNSKRLTRKK